European Patent Specification EP 4 543 900 B1, published August 12, 2026. Title: PEPTIDES FOR INTRACELLULAR DELIVERY. Applicant: UNIVERSIDADE DE SANTIAGO DE COMPOSTELA. The sequence listing filed with the application follows.

SEQUENCE LISTING (72 sequences)

SEQ ID NO: 1 - protein, 7 aa, synthetic construct
  MOD_RES 1: note = ACETYLATION
  REGION 1..7: note = Cationic peptide 7.3(L-H)
  MOD_RES 2: note = Native lysine or modified lysine, wherein the modified lysine is a lysine forming an amide bond with a linker through the e-amino group.
  MOD_RES 5: note = Native lysine or modified lysine, wherein the modified lysine is a lysine forming an amide bond with a linker through the e-amino group.
  MOD_RES 6: note = Native lysine or modified lysine, wherein the modified lysine is a lysine forming an amide bond with a linker through the e-amino group.
  MOD_RES 7: note = AMIDATION
RKHRKKH

SEQ ID NO: 2 - protein, 7 aa, synthetic construct
  MOD_RES 1: note = ACETYLATION
  REGION 1..7: note = Cationic peptide V1-7.3(Leu-His)
  MOD_RES 3: note = Native lysine or modified lysine, wherein the modified lysine is a lysine forming an amide bond with a linker through the e-amino group.
  MOD_RES 4: note = Native lysine or modified lysine, wherein the modified lysine is a lysine forming an amide bond with a linker through the e-amino group.
  MOD_RES 5: note = Native lysine or modified lysine, wherein the modified lysine is a lysine forming an amide bond with a linker through the e-amino group.
  MOD_RES 7: note = AMIDATION
RHKKKHR

SEQ ID NO: 3 - protein, 7 aa, synthetic construct
  MOD_RES 1: note = ACETYLATION
  REGION 1..7: note = Cationic peptide V2-7.3(Leu-His)
  MOD_RES 2: note = Native lysine or modified lysine, wherein the modified lysine is a lysine forming an amide bond with a linker through the e-amino group.
  MOD_RES 5: note = Native lysine or modified lysine, wherein the modified lysine is a lysine forming an amide bond with a linker through the e-amino group.
  MOD_RES 6: note = Native lysine or modified lysine, wherein the modified lysine is a lysine forming an amide bond with a linker through the e-amino group.
  MOD_RES 7: note = AMIDATION
RKHHKKR

SEQ ID NO: 4 - skipped

SEQ ID NO: 5 - protein, 9 aa, synthetic construct
  REGION 1..9: note = Peptide
  VARIANT 2: note = Amino acid independently selected from H, reactive basic amino acid residues containing a reactive group and a hydrophobic amino acid, wherein the hydrophobic amino acid is independently selected from A, V, L and I
  VARIANT 3: note = Amino acid independently selected from H, reactive basic amino acid residues containing a reactive group and a hydrophobic amino acid, wherein the hydrophobic amino acid is independently selected from A, V, L and I
  VARIANT 6: note = Amino acid independently selected from H, reactive basic amino acid residues containing a reactive group and a hydrophobic amino acid, wherein the hydrophobic amino acid is independently selected from A, V, L and I
  VARIANT 7: note = Amino acid independently selected from H, reactive basic amino acid residues containing a reactive group and a hydrophobic amino acid, wherein the hydrophobic amino acid is independently selected from A, V, L and I
  VARIANT 9: note = Amino acid independently selected from H, reactive basic amino acid residues containing a reactive group and a hydrophobic amino acid, wherein the hydrophobic amino acid is independently selected from A, V, L and I
RXXRRXXRX

SEQ ID NO: 6 - protein, 13 aa, synthetic construct
  REGION 1..13: note = Peptide
  VARIANT 3: note = Amino acid independently selected from H, reactive basic amino acid residues containing a reactive group and a hydrophobic amino acid, wherein the hydrophobic amino acid is independently selected from A, V, L and I
  VARIANT 4: note = Amino acid independently selected from H, reactive basic amino acid residues containing a reactive group and a hydrophobic amino acid, wherein the hydrophobic amino acid is independently selected from A, V, L and I
  VARIANT 6: note = Amino acid independently selected from H, reactive basic amino acid residues containing a reactive group and a hydrophobic amino acid, wherein the hydrophobic amino acid is independently selected from A, V, L and I
  VARIANT 7: note = Amino acid independently selected from H, reactive basic amino acid residues containing a reactive group and a hydrophobic amino acid, wherein the hydrophobic amino acid is independently selected from A, V, L and I
  VARIANT 10: note = Amino acid independently selected from H, reactive basic amino acid residues containing a reactive group and a hydrophobic amino acid, wherein the hydrophobic amino acid is independently selected from A, V, L and I
  VARIANT 11: note = Amino acid independently selected from H, reactive basic amino acid residues containing a reactive group and a hydrophobic amino acid, wherein the hydrophobic amino acid is independently selected from A, V, L and I
  VARIANT 13: note = Amino acid independently selected from H, reactive basic amino acid residues containing a reactive group and a hydrophobic amino acid, wherein the hydrophobic amino acid is independently selected from A, V, L and I
RRXXRXXRRXXRX

SEQ ID NO: 7 - protein, 17 aa, synthetic construct
  REGION 1..17: note = Peptide
  VARIANT 3: note = Amino acid independently selected from H, reactive basic amino acid residues containing a reactive group and a hydrophobic amino acid, wherein the hydrophobic amino acid is independently selected from A, V, L and I
  VARIANT 4: note = Amino acid independently selected from H, reactive basic amino acid residues containing a reactive group and a hydrophobic amino acid, wherein the hydrophobic amino acid is independently selected from A, V, L and I
  VARIANT 6: note = Amino acid independently selected from H, reactive basic amino acid residues containing a reactive group and a hydrophobic amino acid, wherein the hydrophobic amino acid is independently selected from A, V, L and I
  VARIANT 7: note = Amino acid independently selected from H, reactive basic amino acid residues containing a reactive group and a hydrophobic amino acid, wherein the hydrophobic amino acid is independently selected from A, V, L and I
  VARIANT 10: note = Amino acid independently selected from H, reactive basic amino acid residues containing a reactive group and a hydrophobic amino acid, wherein the hydrophobic amino acid is independently selected from A, V, L and I
  VARIANT 11: note = Amino acid independently selected from H, reactive basic amino acid residues containing a reactive group and a hydrophobic amino acid, wherein the hydrophobic amino acid is independently selected from A, V, L and I
  VARIANT 13: note = Amino acid independently selected from H, reactive basic amino acid residues containing a reactive group and a hydrophobic amino acid, wherein the hydrophobic amino acid is independently selected from A, V, L and I
  VARIANT 14: note = Amino acid independently selected from H, reactive basic amino acid residues containing a reactive group and a hydrophobic amino acid, wherein the hydrophobic amino acid is independently selected from A, V, L and I
  VARIANT 17: note = Amino acid independently selected from H, reactive basic amino acid residues containing a reactive group and a hydrophobic amino acid, wherein the hydrophobic amino acid is independently selected from A, V, L and I
RRXXRXXRRXXRXXRRX

SEQ ID NO: 8 - protein, 21 aa, synthetic construct
  REGION 1..21: note = Peptide
  VARIANT 3: note = Amino acid selected from H, reactive basic amino acid residues containing a reactive group and a hydrophobic amino acid, wherein the hydrophobic amino acid is selected from A, V, L and I
  VARIANT 4: note = Amino acid selected from H, reactive basic amino acid residues containing a reactive group and a hydrophobic amino acid, wherein the hydrophobic amino acid is selected from A, V, L and I
  VARIANT 6: note = Amino acid selected from H, reactive basic amino acid residues containing a reactive group and a hydrophobic amino acid, wherein the hydrophobic amino acid is selected from A, V, L and I
  VARIANT 7: note = Amino acid selected from H, reactive basic amino acid residues containing a reactive group and a hydrophobic amino acid, wherein the hydrophobic amino acid is selected from A, V, L and I
  VARIANT 10: note = Amino acid selected from H, reactive basic amino acid residues containing a reactive group and a hydrophobic amino acid, wherein the hydrophobic amino acid is selected from A, V, L and I
  VARIANT 11: note = Amino acid selected from H, reactive basic amino acid residues containing a reactive group and a hydrophobic amino acid, wherein the hydrophobic amino acid is selected from A, V, L and I
  VARIANT 13: note = Amino acid selected from H, reactive basic amino acid residues containing a reactive group and a hydrophobic amino acid, wherein the hydrophobic amino acid is selected from A, V, L and I
  VARIANT 14: note = Amino acid selected from H, reactive basic amino acid residues containing a reactive group and a hydrophobic amino acid, wherein the hydrophobic amino acid is selected from A, V, L and I
  VARIANT 17: note = Amino acid selected from H, reactive basic amino acid residues containing a reactive group and a hydrophobic amino acid, wherein the hydrophobic amino acid is selected from A, V, L and I
RRXXRXXRRXXRXXRRXRRLL

SEQ ID NO: 9 - skipped

SEQ ID NO: 10 - protein, 13 aa, synthetic construct
  REGION 1..13: note = Peptide
  VARIANT 2: note = Amino acid independently selected from H, reactive basic amino acid residues containing a reactive group and a hydrophobic amino acid, wherein the hydrophobic amino acid is independently selected from A, V, L and I
  VARIANT 3: note = Amino acid independently selected from H, reactive basic amino acid residues containing a reactive group and a hydrophobic amino acid, wherein the hydrophobic amino acid is independently selected from A, V, L and I
  VARIANT 4: note = Amino acid independently selected from H, reactive basic amino acid residues containing a reactive group and a hydrophobic amino acid, wherein the hydrophobic amino acid is independently selected from A, V, L and I
  VARIANT 6: note = Amino acid independently selected from H, reactive basic amino acid residues containing a reactive group and a hydrophobic amino acid, wherein the hydrophobic amino acid is independently selected from A, V, L and I
  VARIANT 7: note = Amino acid independently selected from H, reactive basic amino acid residues containing a reactive group and a hydrophobic amino acid, wherein the hydrophobic amino acid is independently selected from A, V, L and I
  VARIANT 10: note = Amino acid independently selected from H, reactive basic amino acid residues containing a reactive group and a hydrophobic amino acid, wherein the hydrophobic amino acid is independently selected from A, V, L and I
  VARIANT 11: note = Amino acid independently selected from H, reactive basic amino acid residues containing a reactive group and a hydrophobic amino acid, wherein the hydrophobic amino acid is independently selected from A, V, L and I
  VARIANT 13: note = Amino acid independently selected from H, reactive basic amino acid residues containing a reactive group and a hydrophobic amino acid, wherein the hydrophobic amino acid is independently selected from A, V, L and I
RXXXRXXRRXXRX

SEQ ID NO: 11 - protein, 7 aa, synthetic construct
  MOD_RES 1: note = ACETYLATION
  REGION 1..7: note = Cationic peptide 7.3
  MOD_RES 2: note = Native lysine or modified lysine, wherein the modified lysine is a lysine forming an amide bond with a linker through the e-amino group.
  MOD_RES 5: note = Native lysine or modified lysine, wherein the modified lysine is a lysine forming an amide bond with a linker through the e-amino group.
  MOD_RES 6: note = Native lysine or modified lysine, wherein the modified lysine is a lysine forming an amide bond with a linker through the e-amino group.
  MOD_RES 7: note = AMIDATION
RKLRKKL

SEQ ID NO: 12 - protein, 7 aa, synthetic construct
  MOD_RES 1: note = ACETYLATION
  REGION 1..7: note = Cationic peptide 7.3(Leu-Arg)
  MOD_RES 2: note = Native lysine or modified lysine, wherein the modified lysine is a lysine forming an amide bond with a linker through the e-amino group.
  MOD_RES 5: note = Native lysine or modified lysine, wherein the modified lysine is a lysine forming an amide bond with a linker through the e-amino group.
  MOD_RES 6: note = Native lysine or modified lysine, wherein the modified lysine is a lysine forming an amide bond with a linker through the e-amino group.
  MOD_RES 7: note = AMIDATION
RKRRKKR

SEQ ID NO: 13 - protein, 9 aa, synthetic construct
  MOD_RES 1: note = ACETYLATION
  REGION 1..9: note = Cationic peptide 9.3
  MOD_RES 2: note = Native lysine or modified lysine, wherein the modified lysine is a lysine forming an amide bond with a linker through the e-amino group.
  MOD_RES 6: note = Native lysine or modified lysine, wherein the modified lysine is a lysine forming an amide bond with a linker through the e-amino group.
  MOD_RES 9: note = Native lysine or modified lysine, wherein the modified lysine is a lysine forming an amide bond with a linker through the e-amino group.
  MOD_RES 9: note = AMIDATION
RKLRRKLRK

SEQ ID NO: 14 - protein, 13 aa, synthetic construct
  MOD_RES 1: note = ACETYLATION
  REGION 1..13: note = Cationic peptide 13.3
  MOD_RES 4: note = Native lysine or modified lysine, wherein the modified lysine is a lysine forming an amide bond with a linker through the e-amino group.
  MOD_RES 7: note = Native lysine or modified lysine, wherein the modified lysine is a lysine forming an amide bond with a linker through the e-amino group.
  MOD_RES 11: note = Native lysine or modified lysine, wherein the modified lysine is a lysine forming an amide bond with a linker through the e-amino group.
  MOD_RES 13: note = AMIDATION
RRLKRLKRRLKRL

SEQ ID NO: 15 - protein, 13 aa, synthetic construct
  MOD_RES 1: note = ACETYLATION
  REGION 1..13: note = Cationic peptide 13.3(2+1)
  MOD_RES 4: note = Native lysine or modified lysine, wherein the modified lysine is a lysine forming an amide bond with a linker through the e-amino group.
  MOD_RES 6: note = Native lysine or modified lysine, wherein the modified lysine is a lysine forming an amide bond with a linker through the e-amino group.
  MOD_RES 11: note = Native lysine or modified lysine, wherein the modified lysine is a lysine forming an amide bond with a linker through the e-amino group.
  MOD_RES 13: note = AMIDATION
RRLKRKLRRLKRL

SEQ ID NO: 16 - protein, 13 aa, synthetic construct
  MOD_RES 1: note = ACETYLATION
  REGION 1..13: note = Cationic peptide 13.3(3b)
  MOD_RES 3: note = Native lysine or modified lysine, wherein the modified lysine is a lysine forming an amide bond with a linker through the e-amino group.
  MOD_RES 4: note = Native lysine or modified lysine, wherein the modified lysine is a lysine forming an amide bond with a linker through the e-amino group.
  MOD_RES 6: note = Native lysine or modified lysine, wherein the modified lysine is a lysine forming an amide bond with a linker through the e-amino group.
  MOD_RES 13: note = AMIDATION
RRKKRKLRRLLRL

SEQ ID NO: 17 - protein, 13 aa, synthetic construct
  MOD_RES 1: note = ACETYLATION
  REGION 1..13: note = Cationic peptide 13.3(Leu-His)
  MOD_RES 4: note = Native lysine or modified lysine, wherein the modified lysine is a lysine forming an amide bond with a linker through the e-amino group.
  MOD_RES 7: note = Native lysine or modified lysine, wherein the modified lysine is a lysine forming an amide bond with a linker through the e-amino group.
  MOD_RES 11: note = Native lysine or modified lysine, wherein the modified lysine is a lysine forming an amide bond with a linker through the e-amino group.
  MOD_RES 13: note = AMIDATION
RRHKRLKRRLKRL

SEQ ID NO: 18 - protein, 13 aa, synthetic construct
  MOD_RES 1: note = ACETYLATION
  REGION 1..13: note = Cationic peptide 13.3(R-H)
  MOD_RES 4: note = Native lysine or modified lysine, wherein the modified lysine is a lysine forming an amide bond with a linker through the e-amino group.
  MOD_RES 7: note = Native lysine or modified lysine, wherein the modified lysine is a lysine forming an amide bond with a linker through the e-amino group.
  MOD_RES 11: note = Native lysine or modified lysine, wherein the modified lysine is a lysine forming an amide bond with a linker through the e-amino group.
  MOD_RES 13: note = AMIDATION
RHLKRLKRRLKRL

SEQ ID NO: 19 - protein, 13 aa, synthetic construct
  MOD_RES 1: note = ACETYLATION
  REGION 1..13: note = Cationic peptide 13.3(3His)
  MOD_RES 4: note = Native lysine or modified lysine, wherein the modified lysine is a lysine forming an amide bond with a linker through the e-amino group.
  MOD_RES 7: note = Native lysine or modified lysine, wherein the modified lysine is a lysine forming an amide bond with a linker through the e-amino group.
  MOD_RES 11: note = Native lysine or modified lysine, wherein the modified lysine is a lysine forming an amide bond with a linker through the e-amino group.
  MOD_RES 13: note = AMIDATION
RHLKRHKRRLKRH

SEQ ID NO: 20 - skipped

SEQ ID NO: 21 - protein, 17 aa, synthetic construct
  MOD_RES 1: note = ACETYLATION
  REGION 1..17: note = Cationic peptide 17.3
  MOD_RES 4: note = Native lysine or modified lysine, wherein the modified lysine is a lysine forming an amide bond with a linker through the e-amino group.
  MOD_RES 11: note = Native lysine or modified lysine, wherein the modified lysine is a lysine forming an amide bond with a linker through the e-amino group.
  MOD_RES 14: note = Native lysine or modified lysine, wherein the modified lysine is a lysine forming an amide bond with a linker through the e-amino group.
  MOD_RES 17: note = AMIDATION
RRLKRLLRRLKRLKRRL

SEQ ID NO: 22 - skipped

SEQ ID NO: 23 - protein, 21 aa, synthetic construct
  MOD_RES 1: note = ACETYLATION
  REGION 1..21: note = Cationic peptide 21.3
  MOD_RES 4: note = Native lysine or modified lysine, wherein the modified lysine is a lysine forming an amide bond with a linker through the e-amino group.
  MOD_RES 11: note = Native lysine or modified lysine, wherein the modified lysine is a lysine forming an amide bond with a linker through the e-amino group.
  MOD_RES 14: note = Native lysine or modified lysine, wherein the modified lysine is a lysine forming an amide bond with a linker through the e-amino group.
  MOD_RES 21: note = AMIDATION
RRLKRLLRRLKRLKRRLRRLL

SEQ ID NO: 24-25 - skipped (2 entries)

SEQ ID NO: 26 - protein, 7 aa, synthetic construct
  MOD_RES 1: note = ACETYLATION
  REGION 1..7: note = Cationic peptide 7.2
  MOD_RES 2: note = Native lysine or modified lysine, wherein the modified lysine is a lysine forming an amide bond with a linker through the e-amino group.
  MOD_RES 6: note = Native lysine or modified lysine, wherein the modified lysine is a lysine forming an amide bond with a linker through the e-amino group.
  MOD_RES 7: note = AMIDATION
RKLRRKL

SEQ ID NO: 27 - RNA, 3822 nt, synthetic construct
  misc_feature 1..3822: note = Prefusion stabilized SARS-CoV-2 Spike protein mRNA open reading frame sequence
  source 1..3822: mol_type = other RNA
atgttcgtgtttctggtgctgctgcctctggtgtccagccagtgtgtgaacctgaccacaagaacccagctgcctccagcctacaccaacagctttaccagaggcgtgtactaccccgacaaggtgttcagatccagcgtgctgcactctacccaggacctgttcctgcctttcttcagcaacgtgacctggttccacgccatccacgtgtccggcaccaatggcaccaagagattcgacaaccccgtgctgcccttcaacgacggggtgtactttgccagcaccgagaagtccaacatcatcagaggctggatcttcggcaccacactggacagcaagacccagagcctgctgatcgtgaacaacgccaccaacgtggtcatcaaagtgtgcgagttccagttctgcaacgaccccttcctgggcgtctactatcacaagaacaacaagagctggatggaaagcgagttccgggtgtacagcagcgccaacaactgcaccttcgagtacgtgtcccagcctttcctgatggacctggaaggcaagcagggcaacttcaagaacctgcgcgagttcgtgttcaagaacatcgacggctacttcaagatctacagcaagcacacccctatcaacctcgtgcgggatctgcctcagggcttctctgctctggaacccctggtggatctgcccatcggcatcaacatcacccggtttcagacactgctggccctgcacagaagctacctgacacctggcgatagcagcagcggatggacagctggtgccgccgcttactatgtgggctacctgcagcctagaacctttctgctgaagtacaacgagaacggcaccatcaccgacgccgtggattgtgctctggatcctctgagcgagacaaagtgcaccctgaagtccttcaccgtggaaaagggcatctaccagaccagcaacttccgggtgcagcccaccgaatccatcgtgcggttccccaatatcaccaatctgtgccccttcggcgaggtgttcaatgccaccagattcgcctctgtgtacgcctggaaccggaagcggatcagcaattgcgtggccgactactccgtgctgtacaactccgccagcttcagcaccttcaagtgctacggcgtgtcccctaccaagctgaacgacctgtgcttcacaaacgtgtacgccgacagcttcgtgatccggggagatgaagtgcggcagattgcccctggacagacaggcaagatcgccgactacaactacaagctgcccgacgacttcaccggctgtgtgattgcctggaacagcaacaacctggactccaaagtcggcggcaactacaattacctgtaccggctgttccggaagtccaatctgaagcccttcgagcgggacatctccaccgagatctatcaggccggcagcaccccttgtaacggcgtggaaggcttcaactgctacttcccactgcagtcctacggctttcagcccacaaatggcgtgggctatcagccctacagagtggtggtgctgagcttcgaactgctgcatgcccctgccacagtgtgcggccctaagaaaagcaccaatctcgtgaagaacaaatgcgtgaacttcaacttcaacggcctgaccggcaccggcgtgctgacagagagcaacaagaagttcctgccattccagcagtttggccgggatatcgccgataccacagacgccgttagagatccccagacactggaaatcctggacatcaccccttgcagcttcggcggagtgtctgtgatcacccctggcaccaacaccagcaatcaggtggcagtgctgtaccaggacgtgaactgtaccgaagtgcccgtggccattcacgccgatcagctgacacctacatggcgggtgtactccaccggcagcaatgtgtttcagaccagagccggctgtctgatcggagccgagcacgtgaacaatagctacgagtgcgacatccccatcggcgctggcatctgtgccagctaccagacacagacaaacagccccggcagcgccagctctgtggccagccagagcatcattgcctacacaatgtctctgggcgccgagaacagcgtggcctactccaacaactctatcgctatccccaccaacttcaccatcagcgtgaccacagagatcctgcctgtgtccatgaccaagaccagcgtggactgcaccatgtacatctgcggcgattccaccgagtgctccaacctgctgctgcagtacggcagcttctgcacccagctgaatagagccctgacagggatcgccgtggaacaggacaagaacacccaagaggtgttcgcccaagtgaagcagatctacaagacccctcctatcaaggacttcggcggcttcaatttcagccagattctgcccgatcctagcaagcccagcaagcggagcttcatcgaggacctgctgttcaacaaagtgacactggccgacgccggcttcatcaagcagtatggcgattgtctgggcgacattgccgccagggatctgatttgcgcccagaagtttaacggactgacagtgctgcctcctctgctgaccgatgagatgatcgcccagtacacatctgccctgctggccggcacaatcacaagcggctggacatttggagctggcgccgctctgcagatcccctttgctatgcagatggcctaccggttcaacggcatcggagtgacccagaatgtgctgtacgagaaccagaagctgatcgccaaccagttcaacagcgccatcggcaagatccaggacagcctgagcagcacagcaagcgccctgggaaagctgcaggacgtggtcaaccagaatgcccaggcactgaacaccctggtcaagcagctgtcctccaacttcggcgccatcagctctgtgctgaacgatatcctgagcagactggacccgccggaagccgaggtgcagatcgacagactgatcaccggaaggctgcagtccctgcagacctacgttacccagcagctgatcagagccgccgagattagagcctctgccaatctggccgccaccaagatgtctgagtgtgtgctgggccagagcaagagagtggacttttgcggcaagggctaccacctgatgagcttccctcagtctgcccctcacggcgtggtgtttctgcacgtgacatacgtgcccgctcaagagaagaatttcaccaccgctccagccatctgccacgacggcaaagcccactttcctagagaaggcgtgttcgtgtccaacggcacccattggttcgtgacccagcggaacttctacgagccccagatcatcaccaccgacaacaccttcgtgtctggcaactgcgacgtcgtgatcggcattgtgaacaataccgtgtacgaccctctgcagcccgagctggacagcttcaaagaggaactggataagtactttaagaaccacacaagccccgacgtggacctgggcgatatcagcggaatcaatgccagcgtcgtgaacatccagaaagagatcgaccggctgaacgaggtggccaagaatctgaacgagagcctgatcgacctgcaagaactggggaagtacgagcagtacatcaagtggccctggtacatctggctgggctttatcgccggactgattgccatcgtgatggtcacaatcatgctgtgttgcatgaccagctgctgtagctgcctgaagggctgttgtagctgtggcagctgctgcaagttcgacgaggacgattctgagcccgtgctgaagggcgtgaaactgcactacacctga

SEQ ID NO: 28-30 - skipped (3 entries)

SEQ ID NO: 31 - protein, 9 aa, synthetic construct
  MOD_RES 1: note = ACETYLATION
  REGION 1..9: note = Cationic peptide 9.2
  MOD_RES 2: note = Native lysine or modified lysine, wherein the modified lysine is a lysine forming an amide bond with a linker through the e-amino group.
  MOD_RES 9: note = AMIDATION
  MOD_RES 9: note = Native lysine or modified lysine, wherein the modified lysine is a lysine forming an amide bond with a linker through the e-amino group.
RKLRRLLRK

SEQ ID NO: 32-33 - skipped (2 entries)

SEQ ID NO: 34 - protein, 13 aa, synthetic construct
  MOD_RES 1: note = ACETYLATION
  REGION 1..13: note = Cationic peptide 13.2
  MOD_RES 4: note = Native lysine or modified lysine, wherein the modified lysine is a lysine forming an amide bond with a linker through the e-amino group.
  MOD_RES 11: note = Native lysine or modified lysine, wherein the modified lysine is a lysine forming an amide bond with a linker through the e-amino group.
  MOD_RES 13: note = AMIDATION
RRLKRLLRRLKRL

SEQ ID NO: 35-48 - skipped (14 entries)

SEQ ID NO: 49 - protein, 7 aa, synthetic construct
  MOD_RES 1: note = ACETYLATION
  REGION 1..7: note = Cationic peptide
  MOD_RES 2: note = Native lysine or modified lysine, wherein the modified lysine is a lysine forming an amide bond with a linker through the e-amino group
  MOD_RES 4: note = Native lysine or modified lysine, wherein the modified lysine is a lysine forming an amide bond with a linker through the e-amino group.
  MOD_RES 6: note = Native lysine or modified lysine, wherein the modified lysine is a lysine forming an amide bond with a linker through the e-amino group.
  MOD_RES 7: note = AMIDATION
RKHKHKR

SEQ ID NO: 50-51 - skipped (2 entries)

SEQ ID NO: 52 - protein, 7 aa, synthetic construct
  MOD_RES 1: note = ACETYLATION
  REGION 1..7: note = Cationic peptide 7.3(L-H)(K-O)
  MOD_RES 2: note = Native ornithine or modified ornithine wherein the modified ornithine is an ornithine forming an amide bond with a linker through the d-amino group
  MOD_RES 5: note = Native ornithine or modified ornithine wherein the modified ornithine is an ornithine forming an amide bond with a linker through the d-amino group
  MOD_RES 6: note = Native ornithine or modified ornithine wherein the modified ornithine is an ornithine forming an amide bond with a linker through the d-amino group
  MOD_RES 7: note = AMIDATION
RXHRXXH

SEQ ID NO: 53 - protein, 7 aa, synthetic construct
  MOD_RES 1: note = ACETYLATION
  REGION 1..7: note = Cationic peptide R + 7.3(L-H)-H
  MOD_RES 3: note = Native lysine or modified lysine, wherein the modified lysine is a lysine forming an amide bond with a linker through the e-amino group.
  MOD_RES 6: note = Native lysine or modified lysine, wherein the modified lysine is a lysine forming an amide bond with a linker through the e-amino group
  MOD_RES 7: note = Native lysine or modified lysine wherein the modified lysine is a lysine forming an amide bond with a linker through the e-amino group
  MOD_RES 7: note = AMIDATION
RRKHRKK

SEQ ID NO: 54 - protein, 8 aa, synthetic construct
  MOD_RES 1: note = ACETYLATION
  REGION 1..8: note = Cationic peptide R + 7.3(L-H)
  MOD_RES 3: note = Native lysine or modified lysine, wherein the modified lysine is a lysine forming an amide bond with a linker through the e-amino group
  MOD_RES 6: note = Native lysine or modified lysine, wherein the modified lysine is a lysine forming an amide bond with a linker through the e-amino group
  MOD_RES 7: note = Native lysine or modified lysine, wherein the modified lysine is a lysine forming an amide bond with a linker through the e-amino group
  MOD_RES 8: note = AMIDATION
RRKHRKKH

SEQ ID NO: 55 - protein, 7 aa, synthetic construct
  MOD_RES 1: note = ACETYLATION
  REGION 1..7: note = Cationic peptide R + 7.3- L
  MOD_RES 3: note = Native lysine or modified lysine, wherein the modified lysine is a lysine forming an amide bond with a linker through the e-amino group
  MOD_RES 6: note = Native lysine or modified lysine, wherein the modified lysine is a lysine forming an amide bond with a linker through the e-amino group
  MOD_RES 7: note = Native lysine or modified lysine, wherein the modified lysine is a lysine forming an amide bond with a linker through the e-amino group
  MOD_RES 7: note = AMIDATION
RRKLRKK

SEQ ID NO: 56 - protein, 8 aa, synthetic construct
  MOD_RES 1: note = ACETYLATION
  REGION 1..8: note = Cationic peptide R + 7.3
  MOD_RES 3: note = Native lysine or modified lysine, wherein the modified lysine is a lysine forming an amide bond with a linker through the e-amino group
  MOD_RES 6: note = Native lysine or modified lysine, wherein the modified lysine is a lysine forming an amide bond with a linker through the e-amino group
  MOD_RES 7: note = Native lysine or modified lysine, wherein the modified lysine is a lysine forming an amide bond with a linker through the e-amino group
  MOD_RES 8: note = AMIDATION
RRKLRKKL

SEQ ID NO: 57 - protein, 9 aa, synthetic construct
  MOD_RES 1: note = ACETYLATION
  REGION 1..9: note = Cationic peptide RR + 7.3
  MOD_RES 4: note = Native lysine or modified lysine, wherein the modified lysine is a lysine forming an amide bond with a linker through the e-amino group
  MOD_RES 7: note = Native lysine or modified lysine, wherein the modified lysine is a lysine forming an amide bond with a linker through the e-amino group
  MOD_RES 8: note = Native lysine or modified lysine, wherein the modified lysine is a lysine forming an amide bond with a linker through the e-amino group
  MOD_RES 9: note = AMIDATION
RRRKLRKKL

SEQ ID NO: 58 - protein, 7 aa, synthetic construct
  MOD_RES 1: note = ACETYLATION
  REGION 1..7: note = Cationic peptide V3-7.3(L-H)
  MOD_RES 2: note = Native ornithine or modified ornithine wherein the modified ornithine is an ornithine forming an amide bond with a linker through the d-amino group
  MOD_RES 5: note = Native lysine or modified lysine, wherein the modified lysine is a lysine forming an amide bond with a linker through the e-amino group
  MOD_RES 6: note = Native lysine or modified lysine, wherein the modified lysine is a lysine forming an amide bond with a linker through the e-amino group
  MOD_RES 7: note = AMIDATION
RXHRKKH

SEQ ID NO: 59 - protein, 7 aa, synthetic construct
  MOD_RES 1: note = ACETYLATION
  REGION 1..7: note = Cationic peptide V4-7.3(L-H)
  MOD_RES 2: note = Native lysine or modified lysine, wherein the modified lysine is a lysine forming an amide bond with a linker through the e-amino group
  MOD_RES 5: note = Native lysine or modified lysine, wherein the modified lysine is a lysine forming an amide bond with a linker through the e-amino group
  MOD_RES 6: note = Native ornithine or modified ornithine wherein the modified ornithine is an ornithine forming an amide bond with a linker through the d-amino group
  MOD_RES 7: note = AMIDATION
RKHRKXH

SEQ ID NO: 60 - DNA, 22 bp, synthetic construct
  misc_feature 1..22: note = TLR9 agonist CpG (ODN2395)
  modified_base 1..22: mod_base = OTHER; note = bases are phosphorothioates
  source 1..22: mol_type = other DNA
tcgtcgttttcggcgcgcgccg

SEQ ID NO: 61-63 - skipped (3 entries)

SEQ ID NO: 64 - protein, 8 aa, synthetic construct
  REGION 1..8: note = Immunogenic fragment from OVA
SIINFEKL

SEQ ID NO: 65 - protein, 7 aa, synthetic construct
  source 1..7: note = 1
  MOD_RES 1: note = ACETYLATION
  MOD_RES 2: note = Native lysine or modified lysine, wherein the modified lysine is a lysine forming an amide bond with a linker through the e-amino group
  MOD_RES 5: note = Native lysine or modified lysine, wherein the modified lysine is a lysine forming an amide bond with a linker through the e-amino group
  MOD_RES 6: note = Native lysine or modified lysine, wherein the modified lysine is a lysine forming an amide bond with a linker through the e-amino group
  MOD_RES 7: note = AMIDATION
RKIRKKH

SEQ ID NO: 66 - protein, 7 aa, synthetic construct
  MOD_RES 1: note = ACETYLATION
  MOD_RES 2: note = Native lysine or modified lysine, wherein the modified lysine is a lysine forming an amide bond with a linker through the e-amino group
  MOD_RES 5: note = Native lysine or modified lysine, wherein the modified lysine is a lysine forming an amide bond with a linker through the e-amino group
  MOD_RES 6: note = Native lysine or modified lysine, wherein the modified lysine is a lysine forming an amide bond with a linker through the e-amino group
  MOD_RES 7: note = AMIDATION
RKVRKKH

SEQ ID NO: 67 - skipped

SEQ ID NO: 68 - protein, 7 aa, synthetic construct
  MOD_RES 1: note = ACETYLATION
  MOD_RES 2: note = Native lysine or modified lysine, wherein the modified lysine is a lysine forming an amide bond with a linker through the e-amino group
  MOD_RES 5: note = Native lysine or modified lysine, wherein the modified lysine is a lysine forming an amide bond with a linker through the e-amino group
  MOD_RES 6: note = Native lysine or modified lysine, wherein the modified lysine is a lysine forming an amide bond with a linker through the e-amino group
RKHRKKH

SEQ ID NO: 69 - protein, 7 aa, synthetic construct
  MOD_RES 2: note = Native lysine or modified lysine, wherein the modified lysine is a lysine forming an amide bond with a linker through the e-amino group
  MOD_RES 5: note = Native lysine or modified lysine, wherein the modified lysine is a lysine forming an amide bond with a linker through the e-amino group
  MOD_RES 6: note = Native lysine or modified lysine, wherein the modified lysine is a lysine forming an amide bond with a linker through the e-amino group
  MOD_RES 7: note = AMIDATION
RKHRKKH

SEQ ID NO: 70 - protein, 7 aa, synthetic construct
  MOD_RES 1: note = ACETYLATION
  MOD_RES 2: note = Native Dab or modified Dab wherein the modified Dab is a Dab forming an amide bond with a linker through the gamma-amino group
  MOD_RES 5: note = Native Dab or modified Dab wherein the modified Dab is a Dab forming an amide bond with a linker through the gamma-amino group
  MOD_RES 6: note = Native Dab or modified Dab wherein the modified Dab is a Dab forming an amide bond with a linker through the gamma-amino group
  MOD_RES 7: note = AMIDATION
RXHRXXH

SEQ ID NO: 71 - protein, 7 aa, synthetic construct
  MOD_RES 1: note = ACETYLATION
  MOD_RES 2: note = Modified lysine comprising an aminooxy group, particularly aminooxy acetic acid group
  MOD_RES 5: note = Modified lysine comprising an aminooxy group, particularly aminooxy acetic acid group
  MOD_RES 6: note = Modified lysine comprising an aminooxy group, particularly aminooxy acetic acid group
  METAL 7: note = AMIDATION
RKHRKKH

SEQ ID NO: 72 - protein, 7 aa, synthetic construct
  MOD_RES 1: note = ACETYLATION
  MOD_RES 2: note = Modified lysine comprising succinic acid monohydrazide
  MOD_RES 5: note = Modified lysine comprising succinic acid monohydrazide
  MOD_RES 6: note = Modified lysine comprising succinic acid monohydrazide
  MOD_RES 7: note = AMIDATION
RKHRKKH